European Patent Application EP 4 310 196 A2, published January 24, 2024. Title: METHODS AND COMPOSITIONS FOR MANIPULATING NUCLEIC ACIDS. Applicant: LIFE TECHNOLOGIES CORPORATION. Application EP 18808182.2, filed November 7, 2018. The sequence listing filed with the application follows.

SEQUENCE LISTING (7 sequences)

SEQ ID NO: 1 - DNA, 23 bp, synthetic construct
  misc_feature 1..23: note = Synthetic DNA
  source 1..23: mol_type = other DNA
cctctctatgggcagtcggtgat

SEQ ID NO: 2 - DNA, 20 bp, synthetic construct
  misc_feature 1..20: note = Synthetic DNA
  source 1..20: mol_type = other DNA
ccatctcatccctgcgtgtc

SEQ ID NO: 3 - DNA, 20 bp, synthetic construct
  misc_feature 1..20: note = Synthetic DNA
  source 1..20: mol_type = other DNA
cctatcccctgtgtgccttg

SEQ ID NO: 4 - DNA, 25 bp, synthetic construct
  misc_feature 1..25: note = Synthetic DNA
  source 1..25: mol_type = other DNA
acgatccatctcatccctgcgtgtc

SEQ ID NO: 5 - DNA, 39 bp, synthetic construct
  misc_feature 1..39: note = Synthetic DNA
  source 1..39: mol_type = other DNA
tccataaggtcagtaacgatccatctcatccctgcgtgt

SEQ ID NO: 6 - DNA, 61 bp, synthetic construct
  misc_feature 1..61: note = Synthetic DNA
  source 1..61: mol_type = other DNA
cctatcccctgtgtgccttggcagtctcagccactacgcctccgctttcctctctatggaa

SEQ ID NO: 7 - DNA, 34 bp, synthetic construct
  misc_feature 1..34: note = Synthetic DNA
  source 1..34: mol_type = other DNA
attcgagctgttcatctgtatcttgcgctaccaa